European Patent Application EP 4 524 155 A1, published March 19, 2025. Title: Monoclonal Antibody A38 Against Rift Valley Fever Virus and Use. Applicant: ACADEMY OF MEDICAL SCIENCE,PLA. The sequence listing filed with the application follows.

SEQUENCE LISTING (10 sequences)

SEQ ID NO: 1 - protein, 123 aa, Macaca mulatta
QVQLVQELGPGLVKPSETLSLTCAVSGYSISSPYSWGWIRQPPGKGLEWIGGVYSSGEIRHLDPSLKSRVTLSLDTSKNQFSLKLNSVTAADTAVYFCASANGGVAQDAFDFWGQGLRVTVSS

SEQ ID NO: 2 - DNA, 369 bp, Macaca mulatta
  source 1..369: mol_type = other DNA
caggtccagctggtacaggagttgggcccaggactggtgaagccttcggagaccctgtctctcacctgcgctgtctctggttactccatcagcagtccttactcctggggctggatccgccagcccccagggaaggggctggagtggattgggggtgtctacagtagtggtgagattaggcaccttgacccgtccctcaagagtcgagtcaccctgtcattagacacgtccaagaaccagttctccctgaagctgaactctgtgaccgccgcggacacggccgtgtatttctgtgcctccgccaatgggggggtggctcaagatgcttttgatttctggggccaagggctcagggtcaccgtctcttca

SEQ ID NO: 3 - protein, 330 aa, Homo sapiens [sequence omitted]

SEQ ID NO: 4 - DNA, 990 bp, Homo sapiens
  source 1..990: mol_type = other DNA
gctagcaccaagggcccatcggtcttccccctggcaccctcctccaagagcacctctgggggcacagcggccctgggctgcctggtcaaggactacttccccgaaccggtgacggtgtcgtggaactcaggcgccctgaccagcggcgtgcacaccttcccggctgtcctacagtcctcaggactctactccctcagcagcgtggtgaccgtgccctccagcagcttgggcacccagacctacatctgcaacgtgaatcacaagcccagcaacaccaaggtggacaagaaagttgagcccaaatcttgtgacaaaactcacacatgcccaccgtgcccagcacctgaactcctggggggaccgtcagtcttcctcttccccccaaaacccaaggacaccctcatgatctcccggacccctgaggtcacatgcgtggtggtggacgtgagccacgaagaccctgaggtcaagttcaactggtacgtggacggcgtggaggtgcataatgccaagacaaagccgcgggaggagcagtacaacagcacgtaccgtgtggtcagcgtcctcaccgtcctgcaccaggactggctgaatggcaaggagtacaagtgcaaggtctccaacaaagccctcccagcccccatcgagaaaaccatctccaaagccaaagggcagccccgagaaccacaggtgtacaccctgcctccatctcgggatgagctgaccaagaaccaggtcagcctgacctgcctggtcaaaggcttctatcccagcgacatcgccgtggagtgggagagcaatgggcagccggagaacaactacaagaccacgcctcccgtgctggactccgacggctccttcttcctctatagcaagctcaccgtggacaagagcaggtggcagcaggggaacgtcttctcatgctccgtgatgcatgaggctctgcacaaccactacacgcagaagagcctctccctgtctccgggtaaa

SEQ ID NO: 5 - protein, 116 aa, Macaca mulatta
QPVLTQPPSLSAPPGASARLPCTLSSDLSVTSLNIYWYQQKSGSAPRLFLYYYSDSDKQLGPGVPSRVSGSKETSSNTALLFISGLQPEDEADYYCQVYDSSAYVLFGGGTRLTVL

SEQ ID NO: 6 - DNA, 348 bp, Macaca mulatta
  source 1..348: mol_type = other DNA
cagcctgtgctgactcagccaccctccctgtctgcacccccgggagcatcggccagactcccctgcaccctgagtagtgacctcagtgtcactagtttaaatatatactggtaccaacagaagtcagggagcgctcccaggttattcctgtattactactccgactcagacaagcagctgggacctggggtccccagtcgagtctctggctccaaggagacctcaagtaacacagcgttattgttcatctctgggctccagcctgaggacgaggccgattattactgtcaggtgtatgacagtagtgcatatgtgttattcggaggagggacccggctgaccgtccta

SEQ ID NO: 7 - protein, 107 aa, Homo sapiens [sequence omitted]

SEQ ID NO: 8 - DNA, 321 bp, Homo sapiens
  source 1..321: mol_type = other DNA
cggaccgtggcggcgccatctgtcttcatcttcccgccatctgatgagcagttgaaatctggtaccgctagcgttgtgtgcctgctgaataacttctatcccagagaggccaaagtacagtggaaggtggataacgccctccaatcgggtaactcccaggagagtgtcacagagcaggacagcaaggacagcacctacagcctcagcagcaccctgacgctgagcaaagcagactacgagaaacacaaagtctacgcctgcgaagtcacccatcagggcctgagctcgcccgtcacaaagagcttcaacaggggagagtgt

SEQ ID NO: 9 - protein, 106 aa, Homo sapiens
GQPKAAPSVTLFPPSSEELQANKATLVCLISDFYPGAVTVAWKADSSPVKAGVETTTPSKQSNNKYAASSYLSLTPEQWKSHKSYSCQVTHEGSTVEKTVAPTECS

SEQ ID NO: 10 - DNA, 318 bp, Homo sapiens
  source 1..318: mol_type = other DNA
ggtcagcccaaggctgccccctcggtcactctgttcccaccctcgagtgaggagcttcaagccaacaaggccacactggtgtgtctcataagtgacttctacccgggagccgtgacagtggcctggaaggcagatagcagccccgtcaaggcgggagtggagaccaccacaccctccaaacaaagcaacaacaagtacgcggccagcagctacctgagcctgacgcctgagcagtggaagtcccacaaaagctacagctgccaggtcacgcatgaagggagcaccgtggagaagacagtggcccctacagaatgttca